European Patent Application EP 4 215 547 A1, published July 26, 2023. Title: Single-domain antibody targeting 4-1BB, fusion protein thereof, pharmaceutical composition and use thereof. Applicant: BIOTHEUS INC. The sequence listing filed with the application follows.

SEQUENCE LISTING (174 sequences)

SEQ ID NO: 1 - protein, 116 aa, Artificial Sequence
  single-domain antibody
QVQLVESGGGLVPPGESLRLSCAASGAIFRINTGAWYRQAPGKQRELVASLTTYGKTTYADFVKGRFTISRDDARNTVSLQMNSLKPEDTAIYYCHIGPEPRYGYWGQGTQVTVSS

SEQ ID NO: 2 - protein, 116 aa, Artificial Sequence
  single-domain antibody
QVQLVESGGGLVPPGESLRLSCAASGAIFRINTGAWYRQAPGKQRELVASLTTYGKTTYADFVKGRFTISRDDAENTVSLQMNSLKPEDTAIYYCHIGPEPRYGYWGQGTQVTVSS

SEQ ID NO: 3 - protein, 116 aa, Artificial Sequence
  single-domain antibody
QVQLVESGGGLVPPGESLRLSCAASGAIFRINTGAWYRQAPGKQRELVASLTTYGKTTYADFVKGRFTISRDDAKNTVYLQMNSLKPEDTAIYYCHIGPEPRYGYWGQGTQVTVSS

SEQ ID NO: 4 - protein, 121 aa, Artificial Sequence
  single-domain antibody
QVQLQESGGGLVQVGGSLRLSCAASGFTFDDYAIGWFRQAPGKEREGVLCISSSGGSTYYADSVKGRFTISRDNAKNTVYLQMTNLKPEDTAVYLCGAPRDCSLYTGDDYWGQGTQVTVSS

SEQ ID NO: 5 - protein, 127 aa, Artificial Sequence
  single-domain antibody
QVQLQESGGGLVQAGGSLRLSCAASGFTLDYYAIGWFRQAPGKEREGVLCISSSGETTYYSDSVKGRFTISRDNAKNKVYLQMNSLKPEDTAVYYCGAELLGSGEGCYVWSRDGSYWGQGTQVTVSS

SEQ ID NO: 6 - protein, 116 aa, Artificial Sequence
  single-domain antibody
QVQLQESGGGLVPPGESLRLSCAASGAIFRINTGAWYRQAPGKQRELVASLTTYGKTTYADFVKGRFTISRDDAKNTVSLQMNSLKPEDTAIYYCHIGPEPRYGYWGQGTQVTVSS

SEQ ID NO: 7 - protein, 121 aa, Artificial Sequence
  single-domain antibody
QVQLQESGGGLVQVGGSLRLSCAASGFTFDDYAIGWFRQAPGKEREGVLCISSSGGSTYYADSVKGRFTISRDNAKNTVYLQMTNLKPEDTAVYLCGAPRDCSRYSSDDYWGQGTQVTVSS

SEQ ID NO: 8 - protein, 121 aa, Artificial Sequence
  single-domain antibody
QVQLQESGGGLVEPGGSLRLSCAASGFTFDDYAIGWFRQAPGKEREGVLCISSSGGSTYYADSVKGRFTISRDNAKNTVYLQMTNLKPEDTAVYLCGAPRDCSRYSSDDYWGPGTQVTVSS

SEQ ID NO: 9 - protein, 121 aa, Artificial Sequence
  single-domain antibody
EVQLQESGGGLVQAGGSLRLSCAASGFTFDDYAIGWFRQAPGKEREGVLCISSSGGSTYYADSVKGRFTISRDNAKNTVYLQMTNLKPEDTAVYLCGAPRDCSYYTGDDYWGQGTQVTVSS

SEQ ID NO: 10 - protein, 122 aa, Artificial Sequence
  single-domain antibody
QVQLQESGGGLVQPGGSLRLSCAASGFSLGLYAIGWFRQAPGKEREWVSCIMSSDSSAYYADSVKGRFTVSRDNAKNTVYLQMNRLKPEDTAVYYCAAPQSDCFHYSENDYWGQGTQVTVSS

SEQ ID NO: 11 - protein, 121 aa, Artificial Sequence
  single-domain antibody
QVQLQESGGGLVQPGGSLRLSCAASGFTFDDYAIGWFRQAPGKEREGVLCISSSGGSTYYADSVKGRFTISRDNAKNTVYLQMTNLKPEDTAVYLCGAPRDCSRYSSDDYWGQGTQVTVSS

SEQ ID NO: 12 - protein, 121 aa, Artificial Sequence
  single-domain antibody
QVQLQESGGGLVQAGGSLRLSCAASGFTFDDYAIGWFRQAPGKEREGVLCISSSGGSTYYADSVKGRFTISRDNAKNTVYLQMTNLKPEDTAVYLCGAPRDCSRYSSDDYWGQGTQVTVSS

SEQ ID NO: 13 - protein, 122 aa, Artificial Sequence
  single-domain antibody
QVQLQESGGGLVQAGGSLRLSCAASGFSLGLYAIGWFRQAPGKEREWVSCIMSSDSSAYYADSVKGRFTVSRDNAKNTVYLQMNRLKPEDTAVYYCAAPQSDCFHYSENDYWGQGTQVTVSS

SEQ ID NO: 14 - protein, 122 aa, Artificial Sequence
  single-domain antibody
QVQLQESGGGLVQPGGSLRLSCAASGFSLDYYAIGWFRQAPGKEREWVSCIMSSDSSAYYADSVKGRFTISRDNAKNLVYLRMNSLKPEDTAVYYCTAPRSDCFHYGENDYWGQGTQVTVSS

SEQ ID NO: 15 - protein, 122 aa, Artificial Sequence
  single-domain antibody
QVQLQESGGGLVQAGGSLRLSCAASGFSLDYYAIGWFRQAPGKEREWVSCITASDSSAYYADSVKGRFTISRDNAKNTVYLRMNSLKPEDTAVYYCAAPRSDCFHYGENDYWGQGTQVTVSS

SEQ ID NO: 16 - protein, 122 aa, Artificial Sequence
  single-domain antibody
QVQLQESGGGLVQPGGSLRLSCAASGFSLGLYAIAWFRQAPGKEREWVSCIEKSDSSAYYADSVKGRFTVSRDNAKNTVDLQMNRLSPEDTAVYYCAAPQSDCFHYKENDYWGQGTQVTVSS

SEQ ID NO: 17 - protein, 121 aa, Artificial Sequence
  single-domain antibody
QVQLQESGGGLVQVGGSLRLSCAASGFTFDDYAIGWFRQAPGKEREGVLCISSSGGSTYYADSLKGRFTISRDNAKNTVYLQMTNLKPEDTAVYLCGAPRDCSLYTGDDYWGQGTQVTVSS

SEQ ID NO: 18 - protein, 121 aa, Artificial Sequence
  single-domain antibody
QVQLQESGGGLVQPGGSLRLSCAASGFSLGLYAIGWFRQAPGKEREWVSCIMSSDSSAYYADSVKGRFTVSRDNAKNTVYLQMTNLKPEDTAVYLCGAPRDCSRYSSDDYWGQGTQVTVSS

SEQ ID NO: 19 - protein, 121 aa, Artificial Sequence
  single-domain antibody
QVQLQESGGALVQAGGSLRLSCAASGFTFDDYAIGWFRQAPGKEREGVLCISSSGGSTYYADSVKGRFTISRDNAKNTVYLQMTNLKPEDTAVYLCGAPRDCSRYSSDDYWGQGTQVTVSS

SEQ ID NO: 20 - protein, 121 aa, Artificial Sequence
  single-domain antibody
QVQLQESGGGLVQVGGSLRLSCAASGFTFDDYAIGWFRQAPGKEREGVLCISSSGGSTYYADSVKGRFTISRDNAKNTVYLQMTNLKPEDTAVYLCGAPRDCSLYTGDDYWGPGTQVTVSS

SEQ ID NO: 21 - protein, 121 aa, Artificial Sequence
  single-domain antibody
QVQLQESGGGLVQAGGSLRLSCAASGFTFDDYAIGWFRQAPGKEREGVLCISSSGGSTYYADSVKGRFTISRDNAKNTVYLQMTNLKPEDTAVYLCGAPRDCSYYTSDDYWGQGTQVTVSS

SEQ ID NO: 22 - protein, 121 aa, Artificial Sequence
  single-domain antibody
QVQLQESGGALVQPGGSLRLSCAASGFTFDDYAIGWFRQAPGKEREGVLCISSSGGSTYYADSVKGRFTISRDNAKNTVYLQMTNLKPEDTAVYLCGAPRDCSRYSSDDYWGQGTQVTVSS

SEQ ID NO: 23 - protein, 114 aa, Artificial Sequence
  single-domain antibody
QVQLQESGGGLVQAGGSLRLSCAASGSFNAMGWWRQAPGKQREFVAIITRDGSTNLADSVKGRFTISSDNAKNTWFLQMNSLKPEDTAVYYCSASDYGSSLYYWGQGTQVTVSS

SEQ ID NO: 24 - protein, 125 aa, Artificial Sequence
  single-domain antibody
QVQLQESGGGLVQAGGSLRLSCAASGGTFSITAMGWYRQAPGQQRELVAAIASGDGATNYADFVKGRFTISRDNAKNTMFLQMNSLKPEDSAVYYCYARTGYGSSWPMGHEYDYWGQGTQVTVSS

SEQ ID NO: 25 - protein, 115 aa, Artificial Sequence
  single-domain antibody
QVQLQESGGGLVQPGESLRLSCDSGRIFSYNFMGWYRQAPGKQRELVASITWGGTIKYADSVKGRFTISRHDAENTVYLQMNSLKSEDTAVYYCHAATDTGVIYWGQGTQVTVSS

SEQ ID NO: 26 - protein, 119 aa, Artificial Sequence
  single-domain antibody
QVQLQESGGGLVQAGGSLRLSCAASGRTLSGYVMGWFRQASGKERELVAAISSGGSTYYEDSVKGRFTISRDNAKNTMYLQMNSLKPEDTAVYYCAADPRRLTGLYDYWGQGTQVTVSS

SEQ ID NO: 27 - protein, 117 aa, Artificial Sequence
  single-domain antibody
QVQLQESGGGLVEAGGSLRLSCAASGSIFSINVMGWYRQAPGKQRELVAVITSDYSTNYADSVKGRFTISRDNAKNTVYLQMNSLKPEDTAVYHCAATGYGSSPWYWGQGTQVTVSS

SEQ ID NO: 28 - protein, 125 aa, Artificial Sequence
  single-domain antibody
QVQLQESGGGLVQAGDSLRLSCAASGSTFGITAMGWYRQPPGKQRELVAAIIMSDGDTNYQDSVKGRFTISRDNAKNTMYLQMNSLKLEDTAVYYCYARTGYGSGRLMGHEYDYWGQGTQVTVSS

SEQ ID NO: 29 - protein, 125 aa, Artificial Sequence
  single-domain antibody
QVQLQESGGGLVQPGGSLRLSCAASGSTFSISAMGWYRQPPGKQRELVALIIMSDGDTNYQDSVKGRFTISRDNANNTMYLQMNSLKLEDTAVYYCYARTGYGSGRLMGHEYDYWGQGTQVTVSS

SEQ ID NO: 30 - protein, 125 aa, Artificial Sequence
  single-domain antibody
QVQLQESGGGLVQAGGSLKLSCAASGSTFSISAMGWYRQAPGKQRELVAAIVIGDGDTNYADSVKGRFTISRDNAKNTMYLQMNSLKPEDTAVYYCYARTGYGSSWLMGHEYDYWGQGTQVTVSS

SEQ ID NO: 31 - protein, 125 aa, Artificial Sequence
  single-domain antibody
QVQLQESGGGLVQAGGSLRLSCAASGSTFSITAMGWYRQAPGQQRELVAAIASGDGATNYADFVKGRFTISRDNAKNTMFLQMNSLKPEDSAVYYCYARTGYGSSWLMGHEYDYWGQGTQVTVSS

SEQ ID NO: 32 - protein, 125 aa, Artificial Sequence
  single-domain antibody
QVQLQESGGGLVQAGDSLRLSCAASGSTFSITAMGWYRQPPGKQRELVAAIIMSDGDTNYQDSVKGRFTISRDNAKNTMYLQMNSLKLEDTAVYYCYARTGYGSGRLMGHEYDYWGQGTQVTVSS

SEQ ID NO: 33 - protein, 125 aa, Artificial Sequence
  single-domain antibody
QVQLQESGGGLVQAGDSLRLSCAASGSTFSITAMGWYRQPPGKQRELVAAIIMSDGDTNYQDSVKGRFTISRDNAKNTMYLQMNSLKPEDTAVYYCYARTGYGSGWLEGHEYDYWGQGTQVTVSS

SEQ ID NO: 34 - protein, 125 aa, Artificial Sequence
  single-domain antibody
QVQLQESGGGLVQAGDSLRLSCAASGSTFSITAMGWYRQPPGKQRELVASIITGDGDTNYADSVKGRFTISRDNAKNTMYLQMNSLKPEDTAVYYCYARTGYGSSWLMGHEYDYWGQGTQVTVSS

SEQ ID NO: 35 - protein, 125 aa, Artificial Sequence
  single-domain antibody
QVQLQESGGGLVQAGDSLRLSCAASGSTFSIVAMGWYRQAPGKQRELVASIITGDGDTNYADSVKGRFTISRDNAKNTMYLQMNSLKPEDTAVYYCYARTGYGSSWLMGHEYDYWGQGTQVTVSS

SEQ ID NO: 36 - protein, 120 aa, Artificial Sequence
  single-domain antibody
QVQLQESGGGLVQAGGSLRLSCAASRSIFSSYVMAWYRQAPGKERELVALIRYGGSTDYADSVKGRFTISRDNSKNTLILQMNSLKPEDTAMYYCAASKSAYIFDDRDYWGQGTQVTVSS

SEQ ID NO: 37 - protein, 116 aa, Artificial Sequence
  single-domain antibody
EVQLVESGGGLVKPGGSLRLSCAASGAIFRINTGAWYRQAPGKQRELVASLTTYGKTTYADFVKGRFTISRDDSKNTLYLQMNSLKTEDTAVYYCHIGPEPRYGYWGQGTLVTVSS

SEQ ID NO: 38 - protein, 116 aa, Artificial Sequence
  single-domain antibody
EVQLVESGGGLVKPGGSLRLSCAASGAIFRINTGAWYRQAPGKGLELVASLTTYGKTTYADFVKGRFTISRDDSKNTLYLQMNSLKTEDTAVYYCHIGPEPRYGYWGQGTLVTVSS

SEQ ID NO: 39 - protein, 125 aa, Artificial Sequence
  single-domain antibody
QVQLVESGGGVVQPGRSLRLSCAASGSTFSIVAMGWYRQAPGKQRELVASIITGDGDTNYADSVKGRFTISRDNSKNTMYLQMNSLKPEDTAVYYCYARTGYGSSWLMGHEYDYWGQGTQVTVSS

SEQ ID NO: 40 - protein, 125 aa, Artificial Sequence
  single-domain antibody
QVQLVESGGGVVQPGRSLRLSCAASGSTFSIVAMGWYRQAPGKGLELVASIITGDGDTNYADSVKGRFTISRDNSKNTMYLQMNSLRAEDTAVYYCYARTGYGSSWLMGHEYDYWGQGTQVTVSS

SEQ ID NO: 41 - protein, 13 aa, Artificial Sequence
  CDR
AASGAIFRINTGA

SEQ ID NO: 42 - protein, 13 aa, Artificial Sequence
  CDR
AASGAIFRINTGA

SEQ ID NO: 43 - protein, 13 aa, Artificial Sequence
  CDR
AASGAIFRINTGA

SEQ ID NO: 44 - protein, 13 aa, Artificial Sequence
  CDR
AASGFTFDDYAIG

SEQ ID NO: 45 - protein, 13 aa, Artificial Sequence
  CDR
AASGFTLDYYAIG

SEQ ID NO: 46 - protein, 13 aa, Artificial Sequence
  CDR
AASGAIFRINTGA

SEQ ID NO: 47 - protein, 13 aa, Artificial Sequence
  CDR
AASGFTFDDYAIG

SEQ ID NO: 48 - protein, 13 aa, Artificial Sequence
  CDR
AASGFTFDDYAIG

SEQ ID NO: 49 - protein, 13 aa, Artificial Sequence
  CDR
AASGFTFDDYAIG

SEQ ID NO: 50 - protein, 13 aa, Artificial Sequence
  CDR
AASGFSLGLYAIG

SEQ ID NO: 51 - protein, 13 aa, Artificial Sequence
  CDR
AASGFTFDDYAIG

SEQ ID NO: 52 - protein, 13 aa, Artificial Sequence
  CDR
AASGFTFDDYAIG

SEQ ID NO: 53 - protein, 13 aa, Artificial Sequence
  CDR
AASGFSLGLYAIG

SEQ ID NO: 54 - protein, 13 aa, Artificial Sequence
  CDR
AASGFSLDYYAIG

SEQ ID NO: 55 - protein, 13 aa, Artificial Sequence
  CDR
AASGFSLDYYAIG

SEQ ID NO: 56 - protein, 13 aa, Artificial Sequence
  CDR
AASGFSLGLYAIA

SEQ ID NO: 57 - protein, 13 aa, Artificial Sequence
  CDR
AASGFTFDDYAIG

SEQ ID NO: 58 - protein, 13 aa, Artificial Sequence
  CDR
AASGFSLGLYAIG

SEQ ID NO: 59 - protein, 13 aa, Artificial Sequence
  CDR
AASGFTFDDYAIG

SEQ ID NO: 60 - protein, 13 aa, Artificial Sequence
  CDR
AASGFTFDDYAIG

SEQ ID NO: 61 - protein, 13 aa, Artificial Sequence
  CDR
AASGFTFDDYAIG

SEQ ID NO: 62 - protein, 13 aa, Artificial Sequence
  CDR
AASGFTFDDYAIG

SEQ ID NO: 63 - protein, 10 aa, Artificial Sequence
  CDR
AASGSFNAMG

SEQ ID NO: 64 - protein, 13 aa, Artificial Sequence
  CDR
AASGGTFSITAMG

SEQ ID NO: 65 - protein, 12 aa, Artificial Sequence
  CDR
DSGRIFSYNFMG

SEQ ID NO: 66 - protein, 13 aa, Artificial Sequence
  CDR
AASGRTLSGYVMG

SEQ ID NO: 67 - protein, 13 aa, Artificial Sequence
  CDR
AASGSIFSINVMG

SEQ ID NO: 68 - protein, 13 aa, Artificial Sequence
  CDR
AASGSTFGITAMG

SEQ ID NO: 69 - protein, 13 aa, Artificial Sequence
  CDR
AASGSTFSISAMG

SEQ ID NO: 70 - protein, 13 aa, Artificial Sequence
  CDR
AASGSTFSISAMG

SEQ ID NO: 71 - protein, 13 aa, Artificial Sequence
  CDR
AASGSTFSITAMG

SEQ ID NO: 72 - protein, 13 aa, Artificial Sequence
  CDR
AASGSTFSITAMG

SEQ ID NO: 73 - protein, 13 aa, Artificial Sequence
  CDR
AASGSTFSITAMG

SEQ ID NO: 74 - protein, 13 aa, Artificial Sequence
  CDR
AASGSTFSITAMG

SEQ ID NO: 75 - protein, 13 aa, Artificial Sequence
  CDR
AASGSTFSIVAMG

SEQ ID NO: 76 - protein, 13 aa, Artificial Sequence
  CDR
AASRSIFSSYVMA

SEQ ID NO: 77 - protein, 13 aa, Artificial Sequence
  CDR
AASGAIFRINTGA

SEQ ID NO: 78 - protein, 13 aa, Artificial Sequence
  CDR
AASGAIFRINTGA

SEQ ID NO: 79 - protein, 13 aa, Artificial Sequence
  CDR
AASGSTFSIVAMG

SEQ ID NO: 80 - protein, 13 aa, Artificial Sequence
  CDR
AASGSTFSIVAMG

SEQ ID NO: 81 - protein, 16 aa, Artificial Sequence
  CDR
SLTTYGKTTYADFVKG

SEQ ID NO: 82 - protein, 16 aa, Artificial Sequence
  CDR
SLTTYGKTTYADFVKG

SEQ ID NO: 83 - protein, 16 aa, Artificial Sequence
  CDR
SLTTYGKTTYADFVKG

SEQ ID NO: 84 - protein, 17 aa, Artificial Sequence
  CDR
CISSSGGSTYYADSVKG

SEQ ID NO: 85 - protein, 17 aa, Artificial Sequence
  CDR
CISSSGETTYYSDSVKG

SEQ ID NO: 86 - protein, 16 aa, Artificial Sequence
  CDR
SLTTYGKTTYADFVKG

SEQ ID NO: 87 - protein, 17 aa, Artificial Sequence
  CDR
CISSSGGSTYYADSVKG

SEQ ID NO: 88 - protein, 17 aa, Artificial Sequence
  CDR
CISSSGGSTYYADSVKG

SEQ ID NO: 89 - protein, 17 aa, Artificial Sequence
  CDR
CISSSGGSTYYADSVKG

SEQ ID NO: 90 - protein, 17 aa, Artificial Sequence
  CDR
CIMSSDSSAYYADSVKG

SEQ ID NO: 91 - protein, 17 aa, Artificial Sequence
  CDR
CISSSGGSTYYADSVKG

SEQ ID NO: 92 - protein, 17 aa, Artificial Sequence
  CDR
CISSSGGSTYYADSVKG

SEQ ID NO: 93 - protein, 17 aa, Artificial Sequence
  CDR
CIMSSDSSAYYADSVKG

SEQ ID NO: 94 - protein, 17 aa, Artificial Sequence
  CDR
CIMSSDSSAYYADSVKG

SEQ ID NO: 95 - protein, 17 aa, Artificial Sequence
  CDR
CITASDSSAYYADSVKG

SEQ ID NO: 96 - protein, 17 aa, Artificial Sequence
  CDR
CIEKSDSSAYYADSVKG

SEQ ID NO: 97 - protein, 17 aa, Artificial Sequence
  CDR
CISSSGGSTYYADSLKG

SEQ ID NO: 98 - protein, 17 aa, Artificial Sequence
  CDR
CIMSSDSSAYYADSVKG

SEQ ID NO: 99 - protein, 17 aa, Artificial Sequence
  CDR
CISSSGGSTYYADSVKG

SEQ ID NO: 100 - protein, 17 aa, Artificial Sequence
  CDR
CISSSGGSTYYADSVKG

SEQ ID NO: 101 - protein, 17 aa, Artificial Sequence
  CDR
CISSSGGSTYYADSVKG

SEQ ID NO: 102 - protein, 17 aa, Artificial Sequence
  CDR
CISSSGGSTYYADSVKG

SEQ ID NO: 103 - protein, 16 aa, Artificial Sequence
  CDR
IITRDGSTNLADSVKG

SEQ ID NO: 104 - protein, 17 aa, Artificial Sequence
  CDR
AIASGDGATNYADFVKG

SEQ ID NO: 105 - protein, 16 aa, Artificial Sequence
  CDR
SITWGGTIKYADSVKG

SEQ ID NO: 106 - protein, 16 aa, Artificial Sequence
  CDR
AISSGGSTYYEDSVKG

SEQ ID NO: 107 - protein, 16 aa, Artificial Sequence
  CDR
VITSDYSTNYADSVKG

SEQ ID NO: 108 - protein, 17 aa, Artificial Sequence
  CDR
AIIMSDGDTNYQDSVKG

SEQ ID NO: 109 - protein, 17 aa, Artificial Sequence
  CDR
LIIMSDGDTNYQDSVKG

SEQ ID NO: 110 - protein, 17 aa, Artificial Sequence
  CDR
AIVIGDGDTNYADSVKG

SEQ ID NO: 111 - protein, 17 aa, Artificial Sequence
  CDR
AIASGDGATNYADFVKG

SEQ ID NO: 112 - protein, 17 aa, Artificial Sequence
  CDR
AIIMSDGDTNYQDSVKG

SEQ ID NO: 113 - protein, 17 aa, Artificial Sequence
  CDR
AIIMSDGDTNYQDSVKG

SEQ ID NO: 114 - protein, 17 aa, Artificial Sequence
  CDR
SIITGDGDTNYADSVKG

SEQ ID NO: 115 - protein, 17 aa, Artificial Sequence
  CDR
SIITGDGDTNYADSVKG

SEQ ID NO: 116 - protein, 16 aa, Artificial Sequence
  CDR
LIRYGGSTDYADSVKG

SEQ ID NO: 117 - protein, 16 aa, Artificial Sequence
  CDR
SLTTYGKTTYADFVKG

SEQ ID NO: 118 - protein, 16 aa, Artificial Sequence
  CDR
SLTTYGKTTYADFVKG

SEQ ID NO: 119 - protein, 17 aa, Artificial Sequence
  CDR
SIITGDGDTNYADSVKG

SEQ ID NO: 120 - protein, 17 aa, Artificial Sequence
  CDR
SIITGDGDTNYADSVKG

SEQ ID NO: 121 - protein, 10 aa, Artificial Sequence
  CDR
HIGPEPRYGY

SEQ ID NO: 122 - protein, 10 aa, Artificial Sequence
  CDR
HIGPEPRYGY

SEQ ID NO: 123 - protein, 10 aa, Artificial Sequence
  CDR
HIGPEPRYGY

SEQ ID NO: 124 - protein, 14 aa, Artificial Sequence
  CDR
GAPRDCSLYTGDDY

SEQ ID NO: 125 - protein, 20 aa, Artificial Sequence
  CDR
GAELLGSGEGCYVWSRDGSY

SEQ ID NO: 126 - protein, 10 aa, Artificial Sequence
  CDR
HIGPEPRYGY

SEQ ID NO: 127 - protein, 14 aa, Artificial Sequence
  CDR
GAPRDCSRYSSDDY

SEQ ID NO: 128 - protein, 14 aa, Artificial Sequence
  CDR
GAPRDCSRYSSDDY

SEQ ID NO: 129 - protein, 14 aa, Artificial Sequence
  CDR
GAPRDCSYYTGDDY

SEQ ID NO: 130 - protein, 15 aa, Artificial Sequence
  CDR
AAPQSDCFHYSENDY

SEQ ID NO: 131 - protein, 14 aa, Artificial Sequence
  CDR
GAPRDCSRYSSDDY

SEQ ID NO: 132 - protein, 14 aa, Artificial Sequence
  CDR
GAPRDCSRYSSDDY

SEQ ID NO: 133 - protein, 15 aa, Artificial Sequence
  CDR
AAPQSDCFHYSENDY

SEQ ID NO: 134 - protein, 15 aa, Artificial Sequence
  CDR
TAPRSDCFHYGENDY

SEQ ID NO: 135 - protein, 15 aa, Artificial Sequence
  CDR
AAPRSDCFHYGENDY

SEQ ID NO: 136 - protein, 15 aa, Artificial Sequence
  CDR
AAPQSDCFHYKENDY

SEQ ID NO: 137 - protein, 14 aa, Artificial Sequence
  CDR
GAPRDCSLYTGDDY

SEQ ID NO: 138 - protein, 14 aa, Artificial Sequence
  CDR
GAPRDCSRYSSDDY

SEQ ID NO: 139 - protein, 14 aa, Artificial Sequence
  CDR
GAPRDCSRYSSDDY

SEQ ID NO: 140 - protein, 14 aa, Artificial Sequence
  CDR
GAPRDCSLYTGDDY

SEQ ID NO: 141 - protein, 14 aa, Artificial Sequence
  CDR
GAPRDCSYYTSDDY

SEQ ID NO: 142 - protein, 14 aa, Artificial Sequence
  CDR
GAPRDCSRYSSDDY

SEQ ID NO: 143 - protein, 11 aa, Artificial Sequence
  CDR
SASDYGSSLYY

SEQ ID NO: 144 - protein, 18 aa, Artificial Sequence
  CDR
YARTGYGSSWPMGHEYDY

SEQ ID NO: 145 - protein, 10 aa, Artificial Sequence
  CDR
HAATDTGVIY

SEQ ID NO: 146 - protein, 13 aa, Artificial Sequence
  CDR
AADPRRLTGLYDY

SEQ ID NO: 147 - protein, 11 aa, Artificial Sequence
  CDR
AATGYGSSPWY

SEQ ID NO: 148 - protein, 18 aa, Artificial Sequence
  CDR
YARTGYGSGRLMGHEYDY

SEQ ID NO: 149 - protein, 18 aa, Artificial Sequence
  CDR
YARTGYGSGRLMGHEYDY

SEQ ID NO: 150 - protein, 18 aa, Artificial Sequence
  CDR
YARTGYGSSWLMGHEYDY

SEQ ID NO: 151 - protein, 18 aa, Artificial Sequence
  CDR
YARTGYGSSWLMGHEYDY

SEQ ID NO: 152 - protein, 18 aa, Artificial Sequence
  CDR
YARTGYGSGRLMGHEYDY

SEQ ID NO: 153 - protein, 18 aa, Artificial Sequence
  CDR
YARTGYGSGWLEGHEYDY

SEQ ID NO: 154 - protein, 18 aa, Artificial Sequence
  CDR
YARTGYGSSWLMGHEYDY

SEQ ID NO: 155 - protein, 18 aa, Artificial Sequence
  CDR
YARTGYGSSWLMGHEYDY

SEQ ID NO: 156 - protein, 14 aa, Artificial Sequence
  CDR
AASKSAYIFDDRDY

SEQ ID NO: 157 - protein, 10 aa, Artificial Sequence
  CDR
HIGPEPRYGY

SEQ ID NO: 158 - protein, 10 aa, Artificial Sequence
  CDR
HIGPEPRYGY

SEQ ID NO: 159 - protein, 18 aa, Artificial Sequence
  CDR
YARTGYGSSWLMGHEYDY

SEQ ID NO: 160 - protein, 18 aa, Artificial Sequence
  CDR
YARTGYGSSWLMGHEYDY

SEQ ID NO: 161 - DNA, 23 bp, Artificial Sequence
  primer
gtcctggctgctcttctacaagg

SEQ ID NO: 162 - DNA, 23 bp, Artificial Sequence
  primer
ggtacgtgctgttgaactgttcc

SEQ ID NO: 163 - DNA, 33 bp, Artificial Sequence
  primer
ctagtgcggccgcctggagacggtgacctgggt

SEQ ID NO: 164 - DNA, 38 bp, Artificial Sequence
  primer
cgcggatcccaggtgcagctgcaggagtctggrggagg

SEQ ID NO: 165 - DNA, 89 bp, Artificial Sequence
  primer
atttttactgctgttttattcgcagcatcctccgcattagctaaaagagaggctgaagcacaggtgcagctgcaggagtctggrggagg

SEQ ID NO: 166 - DNA, 81 bp, Artificial Sequence
  primer
agttgtcagttcctgtgccccccctcctcccgcgccacctccgcccgcacctccgccaccactggagacggtgacctgggt

SEQ ID NO: 167 - protein, 224 aa, Artificial Sequence
  Fc of human IgG1
THTCPPCPAPEAAGGPSVFLFPPKPKDTLMISRTPEVTCVVVDVSHEDPEVKFNWYVDGVEVHNAKTKPREEQYNSTYRVVSVLTVLHQDWLNGKEYKCKVSNKALPAPIEKTISKAKGQPREPQVYTLPPSREEMTKNQVSLTCLVKGFYPSDIAVEWESNGQPENNYKTTPPVLDSDGSFFLYSKLTVDKSRWQQGNVFSCSVMHEALHNHYTQKSLSLSPG

SEQ ID NO: 168 - protein, 140 aa, Artificial Sequence
  human 4-1BB protein
QDPCSNCPAGTFCDNNRNQICSPCPPNSFSSAGGQRTCDICRQCKGVFRTRKECSSTSNAECDCTPGFHCLGAGCSMCEQDCKQGQELTKKGCKDCCFGTFNDQKRGICRPWTNCSLDGKSVLVNGTKERDVVCGPSPLG

SEQ ID NO: 169 - protein, 127 aa, Artificial Sequence
  amino sequence of anti 4-1BB antibody in crystalline complex
QVQLVESGGGVVQPGRSLRLSCAASGSTFSIVAMGWYRQAPGKQRELVASIITGDGDTNYADSVKGRFTISRDNSKNTMYLQMNSLKPEDTAVYYCYARTGYGSSWLMGHEYDYWGQGTQVTVSSLG

SEQ ID NO: 170 - protein, 22 aa, Artificial Sequence
  framwork 1
EVQLVESGGGLVKPGGSLRLSC

SEQ ID NO: 171 - protein, 14 aa, Artificial Sequence
  framwork 2
WYRQAPGKQRELVA

SEQ ID NO: 172 - protein, 14 aa, Artificial Sequence
  framwork 2
WYRQAPGKGLELVA

SEQ ID NO: 173 - protein, 30 aa, Artificial Sequence
  framwork 3
RFTISRDDSKNTLYLQMNSLKTEDTAVYYC

SEQ ID NO: 174 - protein, 11 aa, Artificial Sequence
  framwork 4
WGQGTLVTVSS